European Patent Application EP 4 674 845 A1, published January 7, 2026. Title: NOVEL COMPOUNDS AND THEIR APPLICATIONS. Applicant: SFC CO., LTD. Application KR. The sequence listing filed with the application follows.

SEQUENCE LISTING (3 sequences)

SEQ ID NO: 1 - DNA, 20 bp, synthetic construct
  source 1..20: mol_type = other DNA; note = Real-Time PCR forward primer for BQCV (black queen cell virus) plasmid DNA
gcgggagatgatatggactt

SEQ ID NO: 2 - DNA, 21 bp, synthetic construct
  source 1..21: mol_type = other DNA; note = Real-Time PCR reverse primer for BQCV (black queen cell virus) plasmid DNA
ccgtctgagatgcatgaatac

SEQ ID NO: 3 - DNA, 23 bp, synthetic construct
  source 1..23: mol_type = other DNA; note = Real-Time PCR dual labeled probe for BQCV(black queen cell virus) plasmid DNA
ccatctttatcggtacgccgccc